European Patent Application EP 4 349 855 A1, published April 10, 2024. Title: RECOMBINANT CHIMERIC PROTEIN, USE THEREOF, AND COMPOSITION. Applicant: FUNDAÇÃO OSWALDO CRUZ. The sequence listing filed with the application follows.

SEQUENCE LISTING (1 sequence)

SEQ ID NO: 1 - protein, 573 aa, Artificial Sequence
  recombinant chimeric protein containing T. cruzi TS and ASP-2 immunogenic regions
PKSDQPGSQSSFTAVTIEGMRVMLFTHPLNFKGRWLRDRLNLWLTDNQRIYNVGQVSIGDENSAYSSVLYKDDKLYCLHEINTNEVYSLVFARLVGELRIIKSVLQSWKNWDSHLSSICTPADPAASSSERGCGPAVTTVGLVGFLSGNASQNVWEDAYRCVNASTANAERVPNGLKFAGVGGGALWPVSQQGQNQRYRFANHAFTLVASVTIHEAPRDATPLLGASLDSSGGKHGTPSTPVDSSAHGTPSTTVDSSAHGTPSTPVDSSAGGGAGGSGIVMQNNTLVFPLVVNGKNYPFSSITYSTDNGNNWVFPESISPVGCLDPRITEWETGQILMIVDCGNGQSVYESRDMGTTWTKAVRTLSGVWAISQRGVRSYEIFRVGAIITATIEGRKVMLYTRRGYASGEKEANALYLWVTDNNRTFHVGPVAMDSAVNETLSNALLYSDGNLHLLQQRANEKGSAISLARLTEELKEIESVLRTWAQLDAFFSKSSTPTAGLVGFLSNTSSGGNTWIDEYRCVNATVTKASKVKNGFKFTGPGPMATWLVNSREDNRQYSFVNHRFTLVATVT